European Patent Application EP 4 810 616 A1, published September 23, 2026. Title: 외래 프럭토키나아제 및 비-PTS(Non-PTS) 당 유입 인자를 포함하는 미생물 및 이를 이용하여 Ｌ-아미노산을 생산하는 방법. Applicant: 씨제이제일제당 주식회사. The sequence listing filed with the application follows.

SEQUENCE LISTING (160 sequences)

SEQ ID NO: 1 - DNA, 35 bp, synthetic construct
  source 1..35: mol_type = other DNA
tcgagctcggtacccatacctccgacaagccactg

SEQ ID NO: 2 - DNA, 40 bp, synthetic construct
  source 1..40: mol_type = other DNA
gattgcccagaccacgaagaatagcaacttgaccggggac

SEQ ID NO: 3 - DNA, 40 bp, synthetic construct
  source 1..40: mol_type = other DNA
gtccccggtcaagttgctattcttcgtggtctgggcaatc

SEQ ID NO: 4 - DNA, 35 bp, synthetic construct
  source 1..35: mol_type = other DNA
ctctagaggatccccaaaagcaaaaggcggtacca

SEQ ID NO: 5 - DNA, 19 bp, synthetic construct
  source 1..19: mol_type = other DNA
caggtggtaaaggcatcaa

SEQ ID NO: 6 - DNA, 18 bp, synthetic construct
  source 1..18: mol_type = other DNA
ctctcgtttggttgctgt

SEQ ID NO: 7 - DNA, 36 bp, synthetic construct
  source 1..36: mol_type = other DNA
aattcgagctcggtacccagtggacacggaggattt

SEQ ID NO: 8 - DNA, 40 bp, synthetic construct
  source 1..40: mol_type = other DNA
tggtgaccgcattatggagtactgtttagggtggggataa

SEQ ID NO: 9 - DNA, 40 bp, synthetic construct
  source 1..40: mol_type = other DNA
ttatccccaccctaaacagtactccataatgcggtcacca

SEQ ID NO: 10 - DNA, 39 bp, synthetic construct
  source 1..39: mol_type = other DNA
ggtcgactctagaggatccccgtgtaaagagcaatcggg

SEQ ID NO: 11 - DNA, 915 bp, Escherichia coli
  source 1..915: mol_type = genomic DNA; note = cscK
atgtcagccaaagtatgggttttaggggatgcggtcgtagatctcttgccagaatcagacgggcgcctactgccttgtcctggcggcgcgccagctaacgttgcggtgggaatcgccagattaggcggaacaagtgggtttataggtcgggtgggggatgatccttttggtgcgttaatgcaaagaacgctgctaactgagggagtcgatatcacgtatctgaagcaagatgaatggcaccggacatccacggtgcttgtcgatctgaacgatcaaggggaacgttcatttacgtttatggtccgccccagtgccgatctttttttagagacgacagacttgccctgctggcgacatggcgaatggttacatctctgttcaattgcgttgtctgccgagccttcgcgtaccagcgcatttactgcgatgacggcgatccggcatgccggaggttttgtcagcttcgatcctaatattcgtgaagatctatggcaagacgagcatttgctccgcttgtgtttgcggcaggcgctacaactggcggatgtcgtcaagctctcggaagaagaatggcgacttatcagtggaaaaacacagaacgatcaggatatatgcgccctggcaaaagagtatgagatcgccatgctgttggtgactaaaggtgcagaaggggtggtggtctgttatcgaggacaagttcaccattttgctggaatgtctgtgaattgtgtcgatagcacgggggcgggagatgcgttcgttgccgggttactcacaggtctgtcctctacgggattatctacagatgagagagaaatgcgacgaattatcgatctcgctcaacgttgcggagcgcttgcagtaacggcgaaaggggcaatgacagcgctgccatgtcgacaagaactggaatag

SEQ ID NO: 12 - DNA, 35 bp, synthetic construct
  source 1..35: mol_type = other DNA
cgaaaggaaacactcatgtcagccaaagtatgggt

SEQ ID NO: 13 - DNA, 40 bp, synthetic construct
  source 1..40: mol_type = other DNA
tggtgaccgcattatggagtctattccagttcttgtcgac

SEQ ID NO: 14 - DNA, 318 bp, synthetic construct
  source 1..318: mol_type = other DNA; note = CJ7 promoter
agaaacatcccagcgctactaatagggagcgttgaccttccttccacggaccggtaatcggagtgcctaaaaccgcatgcggcttaggctccaagataggttctgcgcggccgggtaatgcatcttctttagcaacaagttgaggggtaggtgcaaataagaacgacatagaaatcgtctcctttctgtttttaatcaacatacaccaccacctaaaaattccccgaccagcaagttcacagtattcgggcacaatatcgttgccaaaatattgtttcggaatatcatgggatacgtacccaacgaaaggaaacactc

SEQ ID NO: 15 - DNA, 40 bp, synthetic construct
  source 1..40: mol_type = other DNA
ttatccccaccctaaacagtagaaacatcccagcgctact

SEQ ID NO: 16 - DNA, 35 bp, synthetic construct
  source 1..35: mol_type = other DNA
tactttggctgacatgagtgtttcctttcgttggg

SEQ ID NO: 17 - DNA, 18 bp, synthetic construct
  source 1..18: mol_type = other DNA
tttttctcccctcgacct

SEQ ID NO: 18 - DNA, 19 bp, synthetic construct
  source 1..19: mol_type = other DNA
tcctcctttcttcttcaac

SEQ ID NO: 19 - DNA, 909 bp, Escherichia coli
  source 1..909: mol_type = genomic DNA; note = mak
gtgcgtataggtatcgatttaggcggcaccaaaactgaagtgattgcactgggcgatgcaggggagcagttgtaccgccatcgtctgcccacgccgcgtgatgattaccggcagactattgaaacgatcgccacgttggttgatatggcggagcaggcgacggggcagcgcggaacggtaggtatgggcattcctggctcaatttcgccttacaccggtgtggtgaagaatgccaattcaacctggctcaacggtcagccattcgataaagacttaagcgcgaggttgcagcgggaagtgcggctggcaaatgacgctaactgtctggcggtttcagaagcagtagatggcgcggcagcgggagcgcagacggtatttgccgtgattatcggcacgggatgcggcgcgggcgtggcattcaatgggcgggcgcatatcggcggcaatggcacggcaggtgagtggggacacaatccgctaccgtggatggacgaagacgaactgcgttatcgcgaggaagtcccttgttattgcggtaaacaaggttgtattgaaacctttatttcgggcacgggattcgcgatggattatcgtcgtttgagcggacatgcgctgaaaggcagtgaaattatccgcctggttgaagaaagcgatccggtagcggaactggcattgcgtcgctacgagctgcggctggcaaaatcgctggcacatgtcgtgaatattctcgatccggatgtgattgtcctggggggcgggatgagcaatgtagaccgtttatatcaaacggttgggcagttgattaaacaatttgtcttcggcggcgaatgtgaaacgccggtgcgtaaggcgaagcacggtgattccagcggcgtacgcggcgctgcgtggttatggccacaagagtaa

SEQ ID NO: 20 - DNA, 38 bp, synthetic construct
  source 1..38: mol_type = other DNA
cgaaaggaaacactcgtgcgtataggtatcgatttagg

SEQ ID NO: 21 - DNA, 40 bp, synthetic construct
  source 1..40: mol_type = other DNA
tggtgaccgcattatggagtttactcttgtggccataacc

SEQ ID NO: 22 - DNA, 40 bp, synthetic construct
  source 1..40: mol_type = other DNA
aaatcgatacctatacgcacgagtgtttcctttcgttggg

SEQ ID NO: 23 - DNA, 924 bp, Klebsiella pneumoniae
  source 1..924: mol_type = genomic DNA; note = scrk
atgaatggaaaaatctgggtactcggcgatgcggtcgtcgatctcctgcccgatggagagggccgcctgctgcaatgccccggcggcgcgccggccaacgtggcggtcggtgtggcgcggctcggcggtgacagcgggtttatcggccgcgtcggcgacgatcccttcggccgttttatgcttcacaccctggcgcaggagcaagtggatgtgaactatatgcgcctcgatgcggcgcagcgcacctccacggtggtggtcgatctcgatagccacggggagcgcacctttacctttatggtccgtccgagcgccgacctgttccttcagcccgaggatctcccgccgtttgccgccggtcagtggctgcacgtctgctccatcgctctcagcgcggagccgagccgcagcacgacattcgcggcgatggaggcgataaagcgcgccgggggctatgtcagcttcgaccccaatatccgcagcgacctgtggcaggatccgcaggaccttcgcgactgtctcgaccgggcgctggccctcgccgacgccataaaactttcggaagaggagctggcgtttatcatcggcagcgacgacatcgtcagcggcatcgcccggctgaacgcccgcttccagccgacgctactgctggtgacccagggtaaagcgggggtacaggccgccctgcgcgggcaggttagccacttccctgcccgcccggtggtggccgtcgataccaccggcgccggcgatgcctttgtcgccgggctactcgccggcctcgccgcccacggtatcccggacaacctcgcagccctggctcccgacctcgcgctggcgcaaacctgcggcgcgctggccaccaccgccaaaggcgccatgaccgccctgccctacagggacgatcttcagcgctcgctgtga

SEQ ID NO: 24 - DNA, 37 bp, synthetic construct
  source 1..37: mol_type = other DNA
aacgaaaggaaacactcatgaatggaaaaatctgggt

SEQ ID NO: 25 - DNA, 37 bp, synthetic construct
  source 1..37: mol_type = other DNA
gtgaccgcattatggagttcacagcgagcgctgaaga

SEQ ID NO: 26 - DNA, 38 bp, synthetic construct
  source 1..38: mol_type = other DNA
ccagatttttccattcatgagtgtttcctttcgttggg

SEQ ID NO: 27 - DNA, 906 bp, Zymomonas mobilis
  source 1..906: mol_type = genomic DNA; note = frk
atgaaaaacgataaaaaaatttatggatgcattgaaggcggcggaacgaaatttatgctcgcccttattgattctgaccggaagatgctggctgtggaacgtgttccgaccacaacccctgaagaaacgcttggtaaaagtgttgaattcttcaaaaaagcgcttcctcaatacgctgattcttttgcgtcttttggtatcgcgtcatttggtccgctttgcctcgatcgcaaaagcccgaaatggggctatatcaccaataccccgaaacctttctggccgaatacggacgttgtaacgccctttaaagaagcttttggttgcccggttgaaatcgacaccgatgtgaatggcgcagctttggctgaaaacttctggggcgcatcaaaaggcacccatacatctgtttatgtcacggttggcaccggcttcggcggtggcgtactgattgatggtaaaccgattcatggtctggctcaccctgaaatgggtcatggtattccgatccgtcatcctgatgatcgtgatttcgaaggttgctgcccttatcatggcggttgctatgaaggtctcgccagcggcacggctatccgtaaacgttggggcaaggctctgaacgaaatggaaccggccgaatttgaaaaagccagagaaatcattgctttctatttggctcacttcaacgtcacgcttcaggcctttatttcaccggaacgtatcgttttcggcggcggcgttatgcatgttgacggtatgctggcttctgttcgtcgtcagacggctgaaattgccaatagttattttgaaggtgctgacttcgaaaaaattatcgtattaccagggttaggtgatcaggccggtatgatgggtgccttcgccttggcattggctgcagaaaataaataa

SEQ ID NO: 28 - DNA, 41 bp, synthetic construct
  source 1..41: mol_type = other DNA
cgaaaggaaacactcatgaaaaacgataaaaaaatttatgg

SEQ ID NO: 29 - DNA, 38 bp, synthetic construct
  source 1..38: mol_type = other DNA
accgcattatggagtttatttattttctgcagccaatg

SEQ ID NO: 30 - DNA, 34 bp, synthetic construct
  source 1..34: mol_type = other DNA
tttatcgtttttcatgagtgtttcctttcgttgg

SEQ ID NO: 31 - DNA, 35 bp, synthetic construct
  source 1..35: mol_type = other DNA
aattcgagctcggtacccgatggaactacgagact

SEQ ID NO: 32 - DNA, 38 bp, synthetic construct
  source 1..38: mol_type = other DNA
tgacaatcaccgcatccagtactggatattcgagacag

SEQ ID NO: 33 - DNA, 39 bp, synthetic construct
  source 1..39: mol_type = other DNA
ctgtctcgaatatccagtactggatgcggtgattgtcag

SEQ ID NO: 34 - DNA, 34 bp, synthetic construct
  source 1..34: mol_type = other DNA
ggtcgactctagaggatcccctaaccacgacgac

SEQ ID NO: 35 - DNA, 1422 bp, Zymomonas mobilis
  source 1..1422: mol_type = genomic DNA; note = glf
atgagttctgaaagtagtcagggtctagtcacgcgactagccctaatcgctgctataggcggcttgcttttcggttacgattcagcggttatcgctgcaatcggtacaccggttgatatccattttattgcccctcgtcacctgtctgctacggctgcggcttccctttctgggatggtcgttgttgctgttttggtcggttgtgttaccggttctttgctgtctggctggattggtattcgcttcggtcgtcgcggcggattgttgatgagttccatttgtttcgtcgccgccggttttggtgctgcgttaaccgaaaaattatttggaaccggtggttcggctttacaaattttttgctttttccggtttcttgccggtttaggtatcggtgtcgtttcaaccttgaccccaacctatattgctgaaattgctccgccagacaaacgtggtcagatggtttctggtcagcagatggccattgtgacgggtgctttaaccggttatatctttacctggttactggctcatttcggttctatcgattgggttaatgccagtggttggtgctggtctccggcttcagaaggcctgatcggtattgccttcttattgctgctgttaaccgcaccggatacgccgcattggttggtgatgaagggacgtcattccgaggctagcaaaatccttgctcgtctggaaccgcaagccgatcctaatctgacgattcaaaagattaaagctggctttgataaagccatggacaaaagcagcgcaggtttgtttgcttttggtatcaccgttgtttttgccggggtatccgttgctgccttccagcagttggtcggtattaacgccgtgctgtattatgcaccgcagatgttccagaatttaggttttggagctgatacggcattattgcagaccatctctatcggtgttgtgaacttcatcttcaccatgattgcttcccgtgttgttgaccgcttcggccgtaaacctctgcttatttggggtgctctcggtatggctgcaatgatggctgttttaggctgctgtttctggttcaaagtcggtggtgttttgcctttggcttctgtgcttctttatattgcagtctttggcatgtcatggggccctgtctgctgggttgttctgtcagaaatgttcccgagttccatcaagggcgcagctatgcctatcgctgttaccggacaatggttagctaatatcttggttaacttcctgtttaaggttgctgatggttctccagcattgaatcagactttcaaccacggtttctcctatctcgttttcgcagcattaagtatcttaggtggcttgattgttgctcgcttcgtgccggaaaccaaaggtcggagcctggatgaaatcgaggagatgtggcgctcccagaagtag

SEQ ID NO: 36 - DNA, 35 bp, synthetic construct
  source 1..35: mol_type = other DNA
cgaaaggaaacactcatgagttctgaaagtagtca

SEQ ID NO: 37 - DNA, 35 bp, synthetic construct
  source 1..35: mol_type = other DNA
atcaccgcatccagtctacttctgggagcgccaca

SEQ ID NO: 38 - DNA, 35 bp, synthetic construct
  source 1..35: mol_type = other DNA
tctcgaatatccagtagaaacatcccagcgctact

SEQ ID NO: 39 - DNA, 35 bp, synthetic construct
  source 1..35: mol_type = other DNA
actttcagaactcatgagtgtttcctttcgttggg

SEQ ID NO: 40 - DNA, 20 bp, synthetic construct
  source 1..20: mol_type = other DNA
aacaacaccacatctacatc

SEQ ID NO: 41 - DNA, 18 bp, synthetic construct
  source 1..18: mol_type = other DNA
cagccttttccagcacca

SEQ ID NO: 42 - DNA, 1476 bp, Corynebacterium glutamicum
  source 1..1476: mol_type = genomic DNA; note = iolT1
atggctagtaccttcattcaggccgacagccctgaaaaaagtaagaagctgcccccactcacagaaggtccgtatagaaagcggctattctacgttgcactagttgcgacgtttggtgggctgctcttcggctacgacaccggcgtcatcaacggtgcactcaacccgatgacccgcgagctcggactaaccgcgttcaccgagggtgttgtaacttcttccctgctgtttggtgcagcagctggtgcgatgtttttcggtcgcatttccgacaactggggtcgccggaaaacaatcatctcacttgcagtagctttctttgtcggcaccatggtctgcgtgtttgctccatcttttgcagtaatggttgtcggacgtgtgcttcttggactcgcagttggtggcgcttccactgttgtccctgtctacctggctgaacttgctccttttgaaatccgtggctcactggctggccgtaatgagttgatgattgttgttggtcagctcgcagctttcgtcatcaatgcgattattggaaatgtttttggacaccacgatggtgtgtggcgctacatgctggcaattgccgcaatcccagcaattgccctcttctttggaatgctccgagttccagaatccccacgctggcttgttgagcgaggacgcattgatgaggctcgcgcagttcttgaaaccattcgccctcttgaacgtgcccatgcagaagttgctgatgttgagcacctagcaagagaagagcacgccgtttccgagaagtccatgggcttaagggaaattttgtccagcaaatggcttgtacgcatcctcctagtaggtatcggattgggtgtcgcacagcagctgaccggcattaactccatcatgtattacggccaggttgttctcattgaggctggtttctccgaaaatgcagctctgatcgccaacgtggcacctggagttatcgcagttgtcggtgcattcatcgcactgtggatgatggatcgtatcaaccgccgtaccaccctcattaccggttattctctcaccaccattagccacgtattgatcggtatcgcatccatagcattcccagtcggcgatccacttcgcccatacgttattttgaccctagttgtggtcttcgtgggatccatgcagaccttcctcaacgtagccacctgggtcatgctctctgagctcttcccgctggcaatgcgaggtttcgcaatcggtatctcagtgttcttcctctggatcgcaaacgcgttcctcggattgttcttccccaccatcatggaagcagtaggactaaccggaaccttcttcatgttcgccggaatcggtgtggttgccttgatcttcatctacacccaggttcctgaaactcgtggacgtaccttggaggagattgatgaggatgttacttccggtgtcattttcaacaaggacatccgaaaaggaaaggtgcactaa

SEQ ID NO: 43 - DNA, 38 bp, synthetic construct
  source 1..38: mol_type = other DNA
cgaaaggaaacactcatggctagtaccttcattcaggc

SEQ ID NO: 44 - DNA, 36 bp, synthetic construct
  source 1..36: mol_type = other DNA
atcaccgcatccagtttagtgcacctttccttttcg

SEQ ID NO: 45 - DNA, 35 bp, synthetic construct
  source 1..35: mol_type = other DNA
gaaggtactagccatgagtgtttcctttcgttggg

SEQ ID NO: 46 - DNA, 1854 bp, Zygosaccharomyces bailii
  source 1..1854: mol_type = genomic DNA; note = ffz1
atggttaagatagacgcttctgcagatttagattggacgaatttacccccccagcagcgcctgggtaggattatcggtggtaaatacatcaacgacagtgttgatgaggccgggccaatctcggctgaacgtccgctcaccaaagtcgagtgtgacctgcccttaacttacaccgagtctgtcgaaggagatggcagagaatgggttgtgctaacgtttgccccagctgaccctcaggatccttacaactgggctctttctcgtaagtggctttacacttcgcttttgtgtggtatgactcttttcatcggttgtgctaccactgtttactcttcgacaatttccagaatggtcttgtcattcgacagagtggctgaaatcggtcagcttggtttgttcactttcaacatgacttgtgccatcgcgcctttatttttggctcccttctgtgagttggtgggtcgttatgtgatctacgtcggtgcctacttgtgtttctctctgtgtttcatcggtttggcccttggtcgtaacattgccactatccttgtgttgcgtaccttgttgggtcttttcggctgtgtgggtaccatcttggtgggtggtacttttgacgatatgttcaagccagaagacagagccattccaatgtccttgttctcatacatcgccattctcggtactgtgggtgctcctatctacgccggtttcgttgatgaaaacgtcggctggcgttggactgaaggtatccagggtcttgcaaacatcccattgctggttgtgatcgttatattcttccgtgaaacccgtggtggtgtgactttgcgtaagagagcccaattattgcgtaaggataccggtgatgacagatgggtctccagggaagagttggaagctccaggtttgaaggatgccctttacgcttcttcggtcaaagccattcaaatgttgtgcactgagcctgtggtgttcttctttggtttgtggattgccttcgcatggttcattaccttcctgttcttgtctgttatcagtatcactttctctgagggtaagcactgggctgaaggtattgccggtcttccatatatcggtttggtgcttggttgtaccttagcttttggtgccaacttccttcagattagaaagtatgacagcttgagagctaaatctaatggtcctctaccaccagagaaccgtctatacggtgctatgtgtggtgctctgtttttgccaattggtcttttcatctactccttctctcaataccctcgtctccactggatgggacctatggttggattgacctgcatttgttttggtatctttttcatctttgagtcgtgctattcttacacctcagactgctatggtcagagtgcttcctccgccattgctggccaaggtttcatgcgtaacaccttgggtgctgtgtctccattgtttgctcaccagttcttcagaaaagtgcacagtcagtacgctggtttgatttgttcggttgtggctacgggtttgaccttccttccttacattttgttcaagtttggcccaaccatcagagctaagtccaagcgtgccattgtctacccagctgacaacggtgacattcttccagatgctgagcagccatctccagatgacagcgagcagatctcctctccatacgaaaaagaaaggagccaagaggaaggtcacatcgagaacgccaatatcccagaaacaacaacaacgactaatgacgaaaagaacagacagggtggtgcagaacttcattcgagtgacgagagtagtaattcaacagaagatgaggttgaggatgctttgcgtatccagcatgatgatgaataaact

SEQ ID NO: 47 - DNA, 35 bp, synthetic construct
  source 1..35: mol_type = other DNA
cgaaaggaaacactcatggttaagatagacgcttc

SEQ ID NO: 48 - DNA, 35 bp, synthetic construct
  source 1..35: mol_type = other DNA
acaatcaccgcatccagtttattcatcatcatgct

SEQ ID NO: 49 - DNA, 35 bp, synthetic construct
  source 1..35: mol_type = other DNA
gtctatcttaaccatgagtgtttcctttcgttggg

SEQ ID NO: 50 - DNA, 1701 bp, Kluyveromyces lactis
  source 1..1701: mol_type = genomic DNA; note = frt1
atgtctagtaatctgtctgaaaaagcagttgaccagcaaaaagaattcggcttgcttaagagtacgagttctgttgactcggtacacgaagttgaagccggtgtgaaagtcggtgaagatgacgacaattattttttcagtgaagatcaaatcttaacacagattaaggtgtacgaagatgaaattgcaaatactccagttactaagacgctaagacaacgtatgagaagaatggaattttgtgaagtgaacttctcaaataaaacgtatatggttattatgcttggttttttcgcatcatttgcaggtattttgtcaggtgtggatcaatcgaccatttcaggtgccagttatggtatgaaggcatcgttgaaattgacttccgatgaagattccttgatttcctctttaatgcctttgggtgcggtcggtggttctatcttgttaactccattaagtgaatatttcggtagaaaagttgccttagtgatctcatgtattttttataccattggtggtattttgtgtgccgctgctcaggatgttcatacaatgtatgcaggcagattcttgatcggtgttggtgtcggtattgaaggtggtggtgttggtgtttatattgctgaatctgtcccatctaccgtgcgtggttccttagtttcgttgtatcaattcaatattgcccttggtgagttggttggttatgtcattggtgtcattttcttcgatgtcaaaggtggttggagatatatgttaggttcctctttggtattttctaccatcttatttgttggtttattcttcttacctgaatcccctcgttggttgatccacaagggttatgatgtagaagcttataaggtctggcgtagattgagagacacatcggatctaggcaataaaagagaattcttggaaatgaaacatgcagctgaacaagatagacaattgaaagaacaagaatctcgcttcaagagtatgtttgacttgatcttaatcccaagaaatcgtcgtgcattgttatactccattatgatggtctctttgggtcaattgactggtattaacgcaatcatgtattatatgtccacgttgatgggacagatcggtttctctccaaaacaagccgtcgctatgtctatggttggtggtgctgctttgttaataggtaccattccagcaatcctatatatggataaatttggtagacgtccatggtctatgaccattatcggtttctccgtaggtctagttctcgtcggtgttggttatcagatcgatttgaataccaacttggctgctgctgaaggggtttacttaaccggccagattttgtataacatcttctttggtacttatgccactttgacctgggttgttccttctgagtctttctctttggctacaagatcgatcggtatgacgatttgctctgctttcttatacttatgggccttcactgttacttataacttcaacaaaatgaaggacgctttcacatacactggtttgactttaggtttctatggtggtattgctattgttattggtattccataccaattgttgtttatgccagaaaccaaagataaaactttggaagaaatcgatgatatctttgagatgccaactagacaattggtcaaacaaaatttgaagaacttaaaagattacgtttctggtaaccgtaaatctatttaa

SEQ ID NO: 51 - DNA, 35 bp, synthetic construct
  source 1..35: mol_type = other DNA
cgaaaggaaacactcatgtctagtaatctgtctga

SEQ ID NO: 52 - DNA, 35 bp, synthetic construct
  source 1..35: mol_type = other DNA
atcaccgcatccagtttaaatagatttacggttac

SEQ ID NO: 53 - RNA, 35 nt, synthetic construct
  source 1..35: mol_type = other RNA
cagattactagacatgagtgtttcctttcgttggg

SEQ ID NO: 54 - DNA, 1713 bp, Saccharomyces cerevisiae
  source 1..1713: mol_type = genomic DNA; note = hxt6
atgtcacaagacgctgctattgcagagcaaactcctgtggagcatctctctgctgttgactcagcctcccactcggttttatctacaccatcaaacaaggctgaaagagatgaaataaaagcttatggtgaaggtgaagagcacgaacctgtcgttgaaattccaaagagaccagcttctgcctatgtcactgtctctattatgtgtatcatgatcgcctttggtggtttcgttttcggttgggatactggtaccatttctggtttcatcaatcaaaccgatttcatcagaagatttggtatgaagcataaagatggtactaattatttgtctaaggttagaactggtttgattgtctccattttcaacattggttgtgccattggtggtattattctttccaaattgggtgatatgtacggtcgtaaggtgggtttgattgtcgttgttgtcatctacatcatcggtattattattcaaattgcatctatcaacaaatggtaccaatatttcatcggtagaattatttccggtttgggtgttggtggtattgccgttttatctcctatgttgatttctgaagtatccccaaagcatttaaggggtactttagtctcttgctaccaattgatgattactgccggtattttcttgggttactgtaccaacttcggtactaagaactactccaactctgtgcaatggagagttccattaggtttgtgttttgcctgggctttgtttatgattggtggtatgacatttgttccagagtctccacgttatttggctgaagtcggtaagatcgaagaagccaaacgttctattgccgtttctaacaaggttgctgttgatgatccatctgttttggctgaagtcgaagctgtcttggctggtgtagaggcagagaaattagctggtaatgcatcctggggtgaattgtttagtagcaagacaaaggtccttcagcgtttgatcatgggtgctatgattcaatctctacaacaattgacaggtgataactatttcttctactatggtactactattttcaaggctgttggtttgagtgactctttcgaaacctctattgtcttgggtattgttaactttgcttccacctttgttggtatttacgttgttgagagatatggtcgtcgtacttgtttgctatggggtgctgcatccatgactgcttgtatggttgtctatgcttccgtgggtgtcaccagattatggccaaatggtcaagaccaaccatcttccaagggtgctggtaactgtatgattgtctttgcctgtttctatattttctgttttgctactacatgggctccaattccttatgtcgttgtttctgaaactttcccattgagagtcaagtctaaggctatgtctattgctacagctgctaattggttgtggggtttcttgattggtttcttcactccatttattactggtgctattaacttctactacggttacgttttcatgggctgtttggtcttcatgttcttctatgttttgttagttgttccagaaactaagggtttgactttggaagaagtcaacaccatgtgggaagaaggtgttctaccatggaagtctgcctcatgggttccaccatctagaagaggtgccaactacgacgctgaagaaatggctcacgatgataagccattgtacaagagaatgttcagcaccaaataa

SEQ ID NO: 55 - DNA, 35 bp, synthetic construct
  source 1..35: mol_type = other DNA
cgaaaggaaacactcatgtcacaagacgctgctat

SEQ ID NO: 56 - DNA, 35 bp, synthetic construct
  source 1..35: mol_type = other DNA
atcaccgcatccagtttatttggtgctgaacattc

SEQ ID NO: 57 - DNA, 35 bp, synthetic construct
  source 1..35: mol_type = other DNA
agcgtcttgtgacatgagtgtttcctttcgttggg

SEQ ID NO: 58 - DNA, 1695 bp, Zygosaccharomyces rouxii
  source 1..1695: mol_type = genomic DNA; note = fsy1
atgaagttttctacttggcggtccaagaccgaaagtgaagtacaagaggtcagtaattcagttgatgacgtttatgaaaaccctgctgttaaaaaagatgaggaatgcgttgaagatttagaaaaagtttcagacgttgatattagccgtagagctaatattgatgaacaactaaaagagttaaatcgtaaaggagatgaatttaagcgcgatcatggatttttcaataatatgaaaaatttagaatttgaaactaatttcaaaaataaaaaacatatggtactcatgcttggtgtgtttgcttcatttgctggtatactatcaggtattgatcaatctatcatatcaggcgcatccattgaaatgaataaaatgttacacttatcttcacatgaagcttcattagtttcatcattgatgcctttaggtgcggtggcaggttccatcttattgacgccatttagtgaaatgttaggtcgtaaaacatctttggttatttcatgtggattttacacaatgggtgctataatctgtgccgcggcacttaatgttcagaccatgtatgcaggtagatttttcattggtgttggtgttggattggaaggtggtggtattggtgtatacattgcagaatgcgttccatctaccgttaggggtcgtctggtttcactttatcaatttaacattgctcttggtgaattatttggttatatcgtcggtgttatattttttgaagttcatggaggttggagatttatggttggatcatcgttaatcttttctacactattattcattggtttgcttttcttaccagaatcgccacgttggttaatgcataagggccgtgtgggtgaatcatggaacatttggaaaaggttgcgggatgtcagtttggaatctgaacagttggaatttttagagttgatccaagccgctaataacgataaagatttacatgcaaatgaatcaagattccaggcttacttcgatttaattcgtatcccacgtaatcgtcgtgccctaatttttgcatcgatcatgattggtttgggtcaactgacgggtatcaatgcaatcatgtactatatgtctacattgatgggcagaattgggttttccgaaaaaagatctgttgccatgtcaatggtcggtggtgccgcgttgttactcggtacaatacctgcaattctctggatggataaatttggtagacgtacatggtcaatgacaattattatattttccgttggtcttgtcctggtcggtgtcggctatctgatcaatattaatactaatctcgtggcggcagaaggtgtttacttaacgggccaaattctttataacatggcatttggttcgtatgcagcactgacatgggttttaccatctgaatcattttcattgagcactagatctgccggtatgaccgttgcatcagctctgttgtacatctttacctttacagtcacatacaattttgatcgtatgcaagccgctatgacttacaccggtttaacactaggcttttacggtggtattgcagtggttatcggtattccttaccaattacttttcatgccggaaacaaaaaatcggacattagaagagatcgacggtattttcagcagacctacaagggaaattgtcagcgagaatatcatgtggttgaaaagaggtaaactaagctattag

SEQ ID NO: 59 - DNA, 35 bp, synthetic construct
  source 1..35: mol_type = other DNA
cgaaaggaaacactcatgaagttttctacttggcg

SEQ ID NO: 60 - DNA, 35 bp, synthetic construct
  source 1..35: mol_type = other DNA
atcaccgcatccagtctaatagcttagtttacctc

SEQ ID NO: 61 - DNA, 35 bp, synthetic construct
  source 1..35: mol_type = other DNA
agtagaaaacttcatgagtgtttcctttcgttggg

SEQ ID NO: 62 - DNA, 1713 bp, Saccharomyces pastorianus
  source 1..1713: mol_type = genomic DNA; note = fsy1
atgtcacatgttaacgcgtcgtatgcgcattcgcaaggatcctcgacaagcgtttctcgtgtagagatggagaagccagcaacaaaggaagtctttgaagatcctaccccaaaaaagtttgaattggacgatgatgaggccggtaagacatcatctgtattcaatccagacctaaatctagaagaagaagtgagagccttggatgaattaggtgattcattcaaaagagatcgctccttttggggcaaaatgaaagctttggaattcgaagttgaatttgaaaataaaaaaaatatggttttaatgctgggaacttttgcagcatttgctggtattctatctggtatagatcaatctattatctctggtgcttccattggtatgaacaaaatgttgcacctttctacacatgaagcatcactagtttcttctttaatgcctctaggtgctgtcgctggttctatattgctaactccctttagtgaatattttggtcgtaaaaagtctttggctatttcttgtgtcttttacacaattggtgctattgtttgtgcagctgcttctaaccatcacgaaatgtatgctggtagatttttgatcggtgtcggtgttggtttagaaggtggtggtattggtgtatacattgcagaatctgttccgtcttcagttagaggtagtctggtgtccctgtatcaatttaatattgcgctgggcgaattgtttggttatattgttggtgtgattttctttgatgttaagggaggctggagatacatggtcggttcgtcgcttgtgttctcgaccacattgtttattggtttattattcctgcctgaatctccacgttggttgatgcataagggccgtgtcggtgaatcctggaacgtctggaaaagactaagagatgtgaaagaagaaggcaataaaatcgaatttttggaactcagagacgttgcttcgcacgacagagagttacatgcaaacgaatcaagatttcaatcattgtttgatttggtccgtgttccacgtaaccgccgtgctttggtatattcttgtatgatgattggtctgggtcaattaactggtattaatgccatcatgtattacatgtccacgctaatgaagaatattgggttcgatgataaacaatctgtagcaatgtcaatggttggtggtgcagcactattaattggtaccgttcctgctattttatggatggatagatttggtagacgtacatgggcaatgacaatcattatatttatcgttggtttggtgctcgtcggtgtcggctatcaaataaacttgaaaacacacatggcagcagcagaaggtgtgtatttgactggtcaaatcatatataacatggcttttggatcatatgcagcattaacatgggtcctaccttcagagtcattttcattgggaaccagatcagctggtatgacagtgtcttctgctttgctttacttgtttgcctttaccgtgacttacaacttcgaaaaaatgaaagaagcaatgacatatacaggtttaaccttagggttttacggtggtatcgctcttgcaattggtatcccataccaattgctatgtatgccagaaacaaagaatagaactttagaggaaattgatgacatctttgagaagccaacaagtcaaattataaaggagaatattgcatacttgaagaagggccaattgagctattag

SEQ ID NO: 63 - DNA, 35 bp, synthetic construct
  source 1..35: mol_type = other DNA
cgaaaggaaacactcatgtcacatgttaacgcgtc

SEQ ID NO: 64 - DNA, 35 bp, synthetic construct
  source 1..35: mol_type = other DNA
atcaccgcatccagtctaatagctcaattggccct

SEQ ID NO: 65 - DNA, 35 bp, synthetic construct
  source 1..35: mol_type = other DNA
gttaacatgtgacatgagtgtttcctttcgttggg

SEQ ID NO: 66 - protein, 281 aa, synthetic construct
  source 1..281: note = HisG(G233H/T235Q)
MLKIAVPNKGSLSERAMEILAEAGYAGRGDSKSLNVFDEANNVEFFFLRPKDIAIYVAGGQLDLGITGRDLARDSQADVHEVLSLGFGSSTFRYAAPADEEWSIEKLDGKRIATSYPNLVRDDLAARGLSAEVLRLDGAVEVSIKLGVADAIADVVSTGRTLRQQGLAPFGEVLCTSEAVIVGRKDEKVTPEQQILLRRIQGILHAQNFLMLDYNVDRDNLDAATAVTPGLSHPQVSPLARDNWVAVRAMVPRRSANAIMDKLAGLGAEAILASEIRIARI

SEQ ID NO: 67 - DNA, 30 bp, synthetic construct
  source 1..30: mol_type = other DNA
gaggagatcaaaacaatgaagacatttgac

SEQ ID NO: 68 - DNA, 30 bp, synthetic construct
  source 1..30: mol_type = other DNA
agtggggatacctgtgggtgggataagcct

SEQ ID NO: 69 - DNA, 30 bp, synthetic construct
  source 1..30: mol_type = other DNA
ggcttatcccacccacaggtatccccactg

SEQ ID NO: 70 - DNA, 28 bp, synthetic construct
  source 1..28: mol_type = other DNA
actctagaggatccccctagatgcgggc

SEQ ID NO: 71 - DNA, 34 bp, synthetic construct
  source 1..34: mol_type = other DNA
tcgagctcggtacccaccgaactcctgacagagt

SEQ ID NO: 72 - DNA, 30 bp, synthetic construct
  source 1..30: mol_type = other DNA
acatgaagcgcctcggtacattcttccaca

SEQ ID NO: 73 - DNA, 294 bp, synthetic construct
  source 1..294: mol_type = other DNA; note = Pspl13
ggcgcttcatgtcaacaatctttaacgttttcaagttcacaagtcgtgttcaaatggtgacaagattggacactgtgctgaattggcaccaagccctcataaatgatagatctaaatcgaatatcaatatatggtctgtttattggaacgcgtcccagtggctgagacgcatccgctaaagccccaggaaccctgtgcagaaagaacaaataatcgtgaattttggcagcaacagcggggcctggtataattgaaaacgtgcaaaagcatagattattggaggagatcaaaaca

SEQ ID NO: 74 - DNA, 30 bp, synthetic construct
  source 1..30: mol_type = other DNA
aagaatgtaccgaggcgcttcatgtcaaca

SEQ ID NO: 75 - DNA, 30 bp, synthetic construct
  source 1..30: mol_type = other DNA
caaatgtcttcattgttttgatctcctcca

SEQ ID NO: 76 - DNA, 18 bp, synthetic construct
  source 1..18: mol_type = other DNA
agcttttcgacgaatccc

SEQ ID NO: 77 - DNA, 20 bp, synthetic construct
  source 1..20: mol_type = other DNA
ctgcctctcacaagttgaag

SEQ ID NO: 78 - DNA, 30 bp, synthetic construct
  source 1..30: mol_type = other DNA
tcgagctcggtacccattggtgctcggcgc

SEQ ID NO: 79 - DNA, 29 bp, synthetic construct
  source 1..29: mol_type = other DNA
tgggatgtttctgtgttgttagtctagtg

SEQ ID NO: 80 - DNA, 34 bp, synthetic construct
  source 1..34: mol_type = other DNA
tcgagctcggtacccaaccaagtttagatgcgcc

SEQ ID NO: 81 - DNA, 31 bp, synthetic construct
  source 1..31: mol_type = other DNA
gctgggatgtttctgccgatagtttatgtca

SEQ ID NO: 82 - DNA, 35 bp, synthetic construct
  source 1..35: mol_type = other DNA
tcgagctcggtacccggtgacagctcgcgccgcat

SEQ ID NO: 83 - DNA, 32 bp, synthetic construct
  source 1..32: mol_type = other DNA
gcgctgggatgtttctggcgaaaagttctccc

SEQ ID NO: 84 - DNA, 33 bp, synthetic construct
  source 1..33: mol_type = other DNA
tcgagctcggtacccttgatgcctgcatgaagg

SEQ ID NO: 85 - DNA, 31 bp, synthetic construct
  source 1..31: mol_type = other DNA
tgacatgaagcgccgaatattgatcctatct

SEQ ID NO: 86 - DNA, 33 bp, synthetic construct
  source 1..33: mol_type = other DNA
ttcgagctcggtacccaccttcagcaaccactc

SEQ ID NO: 87 - DNA, 29 bp, synthetic construct
  source 1..29: mol_type = other DNA
tgacatgaagcgccgaaaaattcttctct

SEQ ID NO: 88 - DNA, 32 bp, synthetic construct
  source 1..32: mol_type = other DNA
aaaggaaacactcatgagcaaatatgcagacg

SEQ ID NO: 89 - DNA, 31 bp, synthetic construct
  source 1..31: mol_type = other DNA
ctagaggatcccccagccggagagggaggag

SEQ ID NO: 90 - DNA, 30 bp, synthetic construct
  source 1..30: mol_type = other DNA
aaaggaaacactcatgaccaaaactgtcgc

SEQ ID NO: 91 - DNA, 31 bp, synthetic construct
  source 1..31: mol_type = other DNA
ctagaggatccccacctctggaggcgtggtc

SEQ ID NO: 92 - DNA, 34 bp, synthetic construct
  source 1..34: mol_type = other DNA
cgaaaggaaacactcatgttgaatgtcactgacc

SEQ ID NO: 93 - DNA, 32 bp, synthetic construct
  source 1..32: mol_type = other DNA
ctagaggatccccccgtgctcagcctgaggag

SEQ ID NO: 94 - DNA, 33 bp, synthetic construct
  source 1..33: mol_type = other DNA
ggagatcaaaacaatgaccttcactattcttcc

SEQ ID NO: 95 - DNA, 32 bp, synthetic construct
  source 1..32: mol_type = other DNA
ctagaggatccccacgaaacgtgcacaacctt

SEQ ID NO: 96 - DNA, 27 bp, synthetic construct
  source 1..27: mol_type = other DNA
gagatcaaaacaatgactgtcgcacca

SEQ ID NO: 97 - DNA, 32 bp, synthetic construct
  source 1..32: mol_type = other DNA
ctagaggatccccgggtcgcggccgtagtggc

SEQ ID NO: 98 - DNA, 32 bp, synthetic construct
  source 1..32: mol_type = other DNA
actagactaacaacacagaaacatcccagcgc

SEQ ID NO: 99 - DNA, 30 bp, synthetic construct
  source 1..30: mol_type = other DNA
tctgcatatttgctcatgagtgtttccttt

SEQ ID NO: 100 - DNA, 33 bp, synthetic construct
  source 1..33: mol_type = other DNA
acataaactatcggcagaaacatcccagcgcta

SEQ ID NO: 101 - DNA, 30 bp, synthetic construct
  source 1..30: mol_type = other DNA
gacagttttggtcatgagtgtttcctttcg

SEQ ID NO: 102 - DNA, 31 bp, synthetic construct
  source 1..31: mol_type = other DNA
gagaacttttcgccagaaacatcccagcgct

SEQ ID NO: 103 - DNA, 30 bp, synthetic construct
  source 1..30: mol_type = other DNA
agtgacattcaacatgagtgtttcctttcg

SEQ ID NO: 104 - DNA, 29 bp, synthetic construct
  source 1..29: mol_type = other DNA
aggatcaatattcggcgcttcatgtcaac

SEQ ID NO: 105 - DNA, 30 bp, synthetic construct
  source 1..30: mol_type = other DNA
gaatagtgaaggtcattgttttgatctcct

SEQ ID NO: 106 - DNA, 29 bp, synthetic construct
  source 1..29: mol_type = other DNA
gagaagaatttttcggcgcttcatgtcaa

SEQ ID NO: 107 - DNA, 29 bp, synthetic construct
  source 1..29: mol_type = other DNA
tggtgcgacagtcattgttttgatctcct

SEQ ID NO: 108 - DNA, 15 bp, synthetic construct
  source 1..15: mol_type = other DNA
gagcatgcatcaaag

SEQ ID NO: 109 - DNA, 19 bp, synthetic construct
  source 1..19: mol_type = other DNA
agaaatttgatccttataa

SEQ ID NO: 110 - DNA, 17 bp, synthetic construct
  source 1..17: mol_type = other DNA
ttgagagatgcttatcg

SEQ ID NO: 111 - DNA, 20 bp, synthetic construct
  source 1..20: mol_type = other DNA
cacttcagtgcggattccaa

SEQ ID NO: 112 - DNA, 17 bp, synthetic construct
  source 1..17: mol_type = other DNA
agcgggtttaattcagg

SEQ ID NO: 113 - DNA, 18 bp, synthetic construct
  source 1..18: mol_type = other DNA
gtgggtaagggttttcgt

SEQ ID NO: 114 - DNA, 19 bp, synthetic construct
  source 1..19: mol_type = other DNA
cacgaaaatgatcgttttg

SEQ ID NO: 115 - DNA, 18 bp, synthetic construct
  source 1..18: mol_type = other DNA
tatgggattcgatggcca

SEQ ID NO: 116 - DNA, 19 bp, synthetic construct
  source 1..19: mol_type = other DNA
tgtgggaatcgctgggcac

SEQ ID NO: 117 - DNA, 16 bp, synthetic construct
  source 1..16: mol_type = other DNA
cggtcgcccgcatctg

SEQ ID NO: 118 - DNA, 31 bp, synthetic construct
  source 1..31: mol_type = other DNA
ttcgagctcggtacccatgaagtctaccggc

SEQ ID NO: 119 - DNA, 30 bp, synthetic construct
  source 1..30: mol_type = other DNA
gacatgaagcgccgacatctaataaccggg

SEQ ID NO: 120 - DNA, 32 bp, synthetic construct
  source 1..32: mol_type = other DNA
ccgacgaggcctaagaactcattccttctgct

SEQ ID NO: 121 - DNA, 31 bp, synthetic construct
  source 1..31: mol_type = other DNA
ctctagaggatccccttagagtgcattgatc

SEQ ID NO: 122 - DNA, 30 bp, synthetic construct
  source 1..30: mol_type = other DNA
ccggttattagatgtcggcgcttcatgtca

SEQ ID NO: 123 - DNA, 25 bp, synthetic construct
  source 1..25: mol_type = other DNA
ggatgtttctctagatgcgggcgat

SEQ ID NO: 124 - DNA, 29 bp, synthetic construct
  source 1..29: mol_type = other DNA
gcccgcatctagagaaacatcccagcgct

SEQ ID NO: 125 - DNA, 29 bp, synthetic construct
  source 1..29: mol_type = other DNA
agaaggaatgagttcttaggcctcgtcgg

SEQ ID NO: 126 - DNA, 19 bp, synthetic construct
  source 1..19: mol_type = other DNA
ctttcagctttccctcccg

SEQ ID NO: 127 - DNA, 17 bp, synthetic construct
  source 1..17: mol_type = other DNA
gctgtacttttagtaca

SEQ ID NO: 128 - DNA, 35 bp, synthetic construct
  source 1..35: mol_type = other DNA
attcgagctcggtaccccctggcgggctcgctgcc

SEQ ID NO: 129 - DNA, 42 bp, synthetic construct
  source 1..42: mol_type = other DNA
agcgctgggatgtttcttgaccaggaacgccggtgccggact

SEQ ID NO: 130 - DNA, 34 bp, synthetic construct
  source 1..34: mol_type = other DNA
tggcgctcccagaagtagtcttcgtggtctgggc

SEQ ID NO: 131 - DNA, 31 bp, synthetic construct
  source 1..31: mol_type = other DNA
actctagaggatccccatttctaggcccgca

SEQ ID NO: 132 - DNA, 40 bp, synthetic construct
  source 1..40: mol_type = other DNA
ccggcaccggcgttcctggtcaagaaacatcccagcgcta

SEQ ID NO: 133 - DNA, 40 bp, synthetic construct
  source 1..40: mol_type = other DNA
cgctgggatgtttctctattccagttcttgtcgacatggc

SEQ ID NO: 134 - DNA, 32 bp, synthetic construct
  source 1..32: mol_type = other DNA
caagaactggaatagagaaacatcccagcgct

SEQ ID NO: 135 - DNA, 29 bp, synthetic construct
  source 1..29: mol_type = other DNA
agaccacgaagactacttctgggagcgcc

SEQ ID NO: 136 - DNA, 19 bp, synthetic construct
  source 1..19: mol_type = other DNA
caacaagaacgtccgcacc

SEQ ID NO: 137 - DNA, 19 bp, synthetic construct
  source 1..19: mol_type = other DNA
tcgagatccgtgggcactc

SEQ ID NO: 138 - DNA, 5802 bp, synthetic construct
  source 1..5802: mol_type = other DNA; note = pDC24
gttcgcttgctgtccataaaaccgcccagtctagctatcgccatgtaagcccactgcaagctacctgctttctctttgcgcttgcgttttcccttgtccagatagcccagtagctgacattcatccggggtcagcaccgtttctgcggactggctttctacgtgttccgcttcctttagcagcccttgcgccctgagtgcttgcggcagcgtgaagctagcttttatcgccattcgccattcaggctgcgcaactgttgggaagggcgatcggtgcgggcctcttcgctattacgccagctggcgaaagggggatgtgctgcaaggcgattaagttgggtaacgccagggttttcccagtcacgacgttgtaaaacgacggccagtgaattcgagctcggtacccggggatcctctagagtcgacctgcaggcatgcaagcttggcgtaatcatggtcatagctgtttcctgtgtgaaattgttatccgctcacaattccacacaacatacgagccggaagcataaagtgtaaagcctggggtgcctaatgagtgagctaactcacattaattgcgttgcgctcactgcccgctttccagtcgggaaacctgtcgtgccagctgcattaatgaatcggccaacgcgcggggagaggcggtttgcgtattgggcgctcttccgcttcctcgctcactgactcgctgcgctcggtcgttcggctgcggcgagcggtatcagctcactcaaaggcggtaatacggttatccacagaatcaggggataacgcaggaaagaacatgtgagcaaaaggccagcaaaaggccaggaaccgtaaaaaggccgcgttgctggcgtttttccataggctccgcccccctgacgagcatcacaaaaatcgacgctcaagtcagaggtggcgaaacccgacaggactataaagataccaggcgtttccccctggaagctccctcgtgcgctctcctgttccgaccctgccgcttaccggatacctgtccgcctttctcccttcgggaagcgtggcgctttctcaatgctcacgctgtaggtatctcagttcggtgtaggtcgttcgctccaagctgggctgtgtgcacgaaccccccgttcagcccgaccgctgcgccttatccggtaactatcgtcttgagtccaacccggtaagacacgacttatcgccactggcagcagccactggtaacaggattagcagagcgaggtatgtaggcggtgctacagagttcttgaagtggtggcctaactacggctacactagaaggacagtatttggtatctgcgctctgctgaagccagttaccttcggaaaaagagttggtagctcttgatccggcaaacaaaccaccgctggtagcggtggtttttttgtttgcaagcagcagattacgcgcagaaaaaaaggatctcaagaagatcctttgatcttttctacggggtctgacgctcagtggaacgaaaactcacgttaagggattttggtcatgagattatcaaaaaggatcttcacctagatccttttggggtgggcgaagaactccagcatgagatccccgcgctggaggatcatccagccctgatagaaacagaagccactggagcacctcaaaaacaccatcatacactaaatcagtaagttggcagcatcacccgacgcactttgcgccgaataaatacctgtgacggaagatcacttcgcagaataaataaatcctggtgtccctgttgataccgggaagccctgggccaacttttggcgaaaatgagacgttgatcggcacgtaagaggttccaactttcaccataatgaaataagatcactaccgggcgtattttttgagttatcgagattttcaggagctgatagaaacagaagccactggagcacctcaaaaacaccatcatacactaaatcagtaagttggcagcatcacccgacgcactttgcgccgaataaatacctgtgacggaagatcacttcgcagaataaataaatcctggtgtccctgttgataccgggaagccctgggccaacttttggcgaaaatgagacgttgatcggcacgtaagaggttccaactttcaccataatgaaataagatcactaccgggcgtattttttgagttatcgagattttcaggagctctttggcatcgtctctcgcctgtcccctcagttcagtaatttcctgcatttgcctgtttccagtcggtagatattccacaaaacagcagggaagcagcgcttttccgctgcataaccctgcttcggggtcattatagcgattttttcggtatatccatcctttttcgcacgatatacaggattttgccaaagggttcgtgtagactttccttggtgtatccaacggcgtcagccgggcaggataggtgaagtaggcccacccgcgagcgggtgttccttcttcactgtcccttattcgcacctggcggtgctcaacgggaatcctgctctgcgaggctggccggctaccgccggcgtaacagatgagggcaagcggatggctgatgaaaccaagccaaccaggaagggcagcccacctatcaaggtgtactgccttccagacgaacgaagagcgattgaggaaaaggcggcggcggccggcatgagcctgtcggcctacctgctggccgtcggccagggctacaaaatcacgggcgtcgtggactatgagcacgtccgcgagggcgtcccggaaaacgattccgaagcccaacctttcatagaaggcggcggtggaatcgaaatctcgtgatggcaggttgggcgtcgcttggtcggtcatttcgaaaaaggttaggaatacggttagccatttgcctgcttttatatagttcatatgggattcacctttatgttgataagaaataaaagaaaatgccaataggatatcggcattttcttttgcgtttttatttgttaactgttaattgtccttgttcaaggatgctgtctttgacaacagatgttttcttgcctttgatgttcagcaggaagctcggcgcaaacgttgattgtttgtctgcgtagaatcctctgtttgtcatatagcttgtaatcacgacattgtttcctttcgcttgaggtacagcgaagtgtgagtaagtaaaggttacatcgttaggcggatcaagatccatttttaacacaaggccagttttgttcagcggcttgtatgggccagttaaagaattagaaacataaccaagcatgtaaatatcgttagacgtaatgccgtcaatcgtcatttttgatccgcgggagtcagtgaacaggtaccatttgccgttcattttaaagacgttcgcgcgttcaatttcatctgttactgtgttagatgcaatcagcggtttcatcacttttttcagtgtgtaatcatcgtttagctcaatcataccgagagcgccgtttgctaactcagccgtgcgttttttatcgctttgcagaagtttttgactttcttgacggaagaatgatgtgcttttgccatagtatgctttgttaaataaagattcttcgccttggtagccatcttcagttccagtgtttgcttcaaatactaagtatttgtggcctttatcttctacgtagtgaggatctctcagcgtatggttgtcgcctgagctgtagttgccttcatcgatgaactgctgtacattttgatacgtttttccgtcaccgtcaaagattgatttataatcctctacaccgttgatgttcaaagagctgtctgatgctgatacgttaacttgtgcagttgtcagtgtttgtttgccgtaatgtttaccggagaaatcagtgtagaataaacggatttttccgtcagatgtaaatgtggctgaacctgaccattcttgtgtttggtcttttaggatagaatcatttgcatcgaatttgtcgctgtctttaaagacgcggccagcgtttttccagctgtcaatagaagtttcgccgactttttgatagaacatgtaaatcgatgtgtcatccgcatttttaggatctccggctaatgcaaagacgatgtggtagccgtgatagtttgcgacagtgccgtcagcgttttgtaatggccagctgtcccaaacgtccaggccttttgcagaagagatatttttaattgtggacgaatcaaattcagaaacttgatatttttcatttttttgctgttcagggatttgcagcatatcatggcgtgtaatatgggaaatgccgtatgtttccttatatggcttttggttcgtttctttcgcaaacgcttgagttgcgcctcctgccagcagtgcggtagtaaaggttaatactgttgcttgttttgcaaactttttgatgttcatcgttcatgtctccttttttatgtactgtgttagcggtctgcttcttccagccctcctgtttgaagatggcaagttagttacgcacaataaaaaaagacctaaaatatgtaaggggtgacgccaaagtatacactttgccctttacacattttaggtcttgcctgctttatcagtaacaaacccgcgcgatttacttttcgacctcattctattagactctcgtttggattgcaactggtctattttcctcttttgtttgatagaaaatcataaaaggatttgcagactacgggcctaaagaactaaaaaatctatctgtttcttttcattctctgtattttttatagtttctgttgcatgggcataaagttgcctttttaatcacaattcagaaaatatcataatatctcatttcactaaataatagtgaacggcaggtatatgtgatgggttaaaaaggatcaccccagagtcccgctcagaagaactcgtcaagaaggcgatagaaggcgatgcgctgcgaatcgggagcggcgataccgtaaagcacgaggaagcggtcagcccattcgccgccaagctcttcagcaatatcacgggtagccaacgctatgtcctgatagcggtccgccacacccagccggccacagtcgatgaatccagaaaagcggccattttccaccatgatattcggcaagcaggcatcgccatgggtcacgacgagatcctcgccgtcgggcatccgcgccttgagcctggcgaacagttcggctggcgcgagcccctgatgctcttcgtccagatcatcctgatcgacaagaccggcttccatccgagtacgtgctcgctcgatgcgatgtttcgcttggtggtcgaatgggcaggtagccggatcaagcgtatgcagccgccgcattgcatcagccatgatggatactttctcggcaggagcaaggtgagatgacaggagatcctgccccggcacttcgcccaatagcagccagtcccttcccgcttcagtgacaacgtcgagacagctgcgcaaggaacgcccgtcgtggccagccacgatagccgcgctgcctcgtcttggagttcattcagggcaccggacaggtcggtcttgacaaaaagaaccgggcgcccctgcgctgacagccggaacacggcggcatcagagcagccgattgtctgttgtgcccagtcatagccgaatagcctctccacccaagcggccggagaacctgcgtgcaatccatcttgttcaatcatgcgaaacgatcctcatcctgtctcttgatcagatcttgatcccctgcgccatcagatccttggcggcaagaaagccatccagtttactttgcagggcttcccaaccttaccagagggcgccccagctggcaattccg

SEQ ID NO: 139 - protein, 304 aa, Escherichia coli
  source 1..304: note = cscK
MSAKVWVLGDAVVDLLPESDGRLLPCPGGAPANVAVGIARLGGTSGFIGRVGDDPFGALMQRTLLTEGVDITYLKQDEWHRTSTVLVDLNDQGERSFTFMVRPSADLFLETTDLPCWRHGEWLHLCSIALSAEPSRTSAFTAMTAIRHAGGFVSFDPNIREDLWQDEHLLRLCLRQALQLADVVKLSEEEWRLISGKTQNDQDICALAKEYEIAMLLVTKGAEGVVVCYRGQVHHFAGMSVNCVDSTGAGDAFVAGLLTGLSSTGLSTDEREMRRIIDLAQRCGALAVTAKGAMTALPCRQELE

SEQ ID NO: 140 - protein, 473 aa, Zymomonas mobilis
  source 1..473: note = glf
MSSESSQGLVTRLALIAAIGGLLFGYDSAVIAAIGTPVDIHFIAPRHLSATAAASLSGMVVVAVLVGCVTGSLLSGWIGIRFGRRGGLLMSSICFVAAGFGAALTEKLFGTGGSALQIFCFFRFLAGLGIGVVSTLTPTYIAEIAPPDKRGQMVSGQQMAIVTGALTGYIFTWLLAHFGSIDWVNASGWCWSPASEGLIGIAFLLLLLTAPDTPHWLVMKGRHSEASKILARLEPQADPNLTIQKIKAGFDKAMDKSSAGLFAFGITVVFAGVSVAAFQQLVGINAVLYYAPQMFQNLGFGADTALLQTISIGVVNFIFTMIASRVVDRFGRKPLLIWGALGMAAMMAVLGCCFWFKVGGVLPLASVLLYIAVFGMSWGPVCWVVLSEMFPSSIKGAAMPIAVTGQWLANILVNFLFKVADGSPALNQTFNHGFSYLVFAALSILGGLIVARFVPETKGRSLDEIEEMWRSQK

SEQ ID NO: 141 - DNA, 30 bp, synthetic construct
  source 1..30: mol_type = other DNA
tcgagctcggtacccccaccacctaaaaat

SEQ ID NO: 142 - DNA, 30 bp, synthetic construct
  source 1..30: mol_type = other DNA
cgtggatgtccggtgacattcatcttgctt

SEQ ID NO: 143 - DNA, 30 bp, synthetic construct
  source 1..30: mol_type = other DNA
ctgaagcaagatgaatgtcaccggacatcc

SEQ ID NO: 144 - DNA, 33 bp, synthetic construct
  source 1..33: mol_type = other DNA
ctctagaggatccccgataattcgtcgcatttc

SEQ ID NO: 145 - DNA, 31 bp, synthetic construct
  source 1..31: mol_type = other DNA
agagcttgacgacatccaccagttgtagcgc

SEQ ID NO: 146 - DNA, 31 bp, synthetic construct
  source 1..31: mol_type = other DNA
gcgctacaactggtggatgtcgtcaagctct

SEQ ID NO: 147 - protein, 304 aa, synthetic construct
MSAKVWVLGDAVVDLLPESDGRLLPCPGGAPANVAVGIARLGGTSGFIGRVGDDPFGALMQRTLLTEGVDITYLKQDECHRTSTVLVDLNDQGERSFTFMVRPSADLFLETTDLPCWRHGEWLHLCSIALSAEPSRTSAFTAMTAIRHAGGFVSFDPNIREDLWQDEHLLRLCLRQALQLADVVKLSEEEWRLISGKTQNDQDICALAKEYEIAMLLVTKGAEGVVVCYRGQVHHFAGMSVNCVDSTGAGDAFVAGLLTGLSSTGLSTDEREMRRIIDLAQRCGALAVTAKGAMTALPCRQELE

SEQ ID NO: 148 - protein, 304 aa, synthetic construct
MSAKVWVLGDAVVDLLPESDGRLLPCPGGAPANVAVGIARLGGTSGFIGRVGDDPFGALMQRTLLTEGVDITYLKQDECHRTSTVLVDLNDQGERSFTFMVRPSADLFLETTDLPCWRHGEWLHLCSIALSAEPSRTSAFTAMTAIRHAGGFVSFDPNIREDLWQDEHLLRLCLRQALQLVDVVKLSEEEWRLISGKTQNDQDICALAKEYEIAMLLVTKGAEGVVVCYRGQVHHFAGMSVNCVDSTGAGDAFVAGLLTGLSSTGLSTDEREMRRIIDLAQRCGALAVTAKGAMTALPCRQELE

SEQ ID NO: 149 - DNA, 915 bp, synthetic construct
  source 1..915: mol_type = other DNA
atgtcagccaaagtatgggttttaggggatgcggtcgtagatctcttgccagaatcagacgggcgcctactgccttgtcctggcggcgcgccagctaacgttgcggtgggaatcgccagattaggcggaacaagtgggtttataggtcgggtgggggatgatccttttggtgcgttaatgcaaagaacgctgctaactgagggagtcgatatcacgtatctgaagcaagatgaatgtcaccggacatccacggtgcttgtcgatctgaacgatcaaggggaacgttcatttacgtttatggtccgccccagtgccgatctttttttagagacgacagacttgccctgctggcgacatggcgaatggttacatctctgttcaattgcgttgtctgccgagccttcgcgtaccagcgcatttactgcgatgacggcgatccggcatgccggaggttttgtcagcttcgatcctaatattcgtgaagatctatggcaagacgagcatttgctccgcttgtgtttgcggcaggcgctacaactggcggatgtcgtcaagctctcggaagaagaatggcgacttatcagtggaaaaacacagaacgatcaggatatatgcgccctggcaaaagagtatgagatcgccatgctgttggtgactaaaggtgcagaaggggtggtggtctgttatcgaggacaagttcaccattttgctggaatgtctgtgaattgtgtcgatagcacgggggcgggagatgcgttcgttgccgggttactcacaggtctgtcctctacgggattatctacagatgagagagaaatgcgacgaattatcgatctcgctcaacgttgcggagcgcttgcagtaacggcgaaaggggcaatgacagcgctgccatgtcgacaagaactggaatag

SEQ ID NO: 150 - DNA, 915 bp, synthetic construct
  source 1..915: mol_type = other DNA
atgtcagccaaagtatgggttttaggggatgcggtcgtagatctcttgccagaatcagacgggcgcctactgccttgtcctggcggcgcgccagctaacgttgcggtgggaatcgccagattaggcggaacaagtgggtttataggtcgggtgggggatgatccttttggtgcgttaatgcaaagaacgctgctaactgagggagtcgatatcacgtatctgaagcaagatgaatgtcaccggacatccacggtgcttgtcgatctgaacgatcaaggggaacgttcatttacgtttatggtccgccccagtgccgatctttttttagagacgacagacttgccctgctggcgacatggcgaatggttacatctctgttcaattgcgttgtctgccgagccttcgcgtaccagcgcatttactgcgatgacggcgatccggcatgccggaggttttgtcagcttcgatcctaatattcgtgaagatctatggcaagacgagcatttgctccgcttgtgtttgcggcaggcgctacaactggtggatgtcgtcaagctctcggaagaagaatggcgacttatcagtggaaaaacacagaacgatcaggatatatgcgccctggcaaaagagtatgagatcgccatgctgttggtgactaaaggtgcagaaggggtggtggtctgttatcgaggacaagttcaccattttgctggaatgtctgtgaattgtgtcgatagcacgggggcgggagatgcgttcgttgccgggttactcacaggtctgtcctctacgggattatctacagatgagagagaaatgcgacgaattatcgatctcgctcaacgttgcggagcgcttgcagtaacggcgaaaggggcaatgacagcgctgccatgtcgacaagaactggaatag

SEQ ID NO: 151 - DNA, 36 bp, synthetic construct
  source 1..36: mol_type = other DNA
ttcgagctcggtaccccaaatgctccaaccgtccgt

SEQ ID NO: 152 - DNA, 33 bp, synthetic construct
  source 1..33: mol_type = other DNA
cgctgggatgtttctgaactcattccttctgct

SEQ ID NO: 153 - DNA, 34 bp, synthetic construct
  source 1..34: mol_type = other DNA
acaagaactggaataggacatctaataaccgggc

SEQ ID NO: 154 - DNA, 34 bp, synthetic construct
  source 1..34: mol_type = other DNA
ctctagaggatcccctacacctccacctgcccag

SEQ ID NO: 155 - DNA, 40 bp, synthetic construct
  source 1..40: mol_type = other DNA
cccaacgaaaggaaacactcatgtcagccaaagtatgggt

SEQ ID NO: 156 - DNA, 36 bp, synthetic construct
  source 1..36: mol_type = other DNA
tgcccggttattagatgtcctattccagttcttgtc

SEQ ID NO: 157 - DNA, 23 bp, synthetic construct
  source 1..23: mol_type = other DNA
atgtccggtgacattcatcttgc

SEQ ID NO: 158 - DNA, 23 bp, synthetic construct
  source 1..23: mol_type = other DNA
aagatgaatgtcaccggacatcc

SEQ ID NO: 159 - DNA, 30 bp, synthetic construct
  source 1..30: mol_type = other DNA
acatccaccagttgtagcgcctgccgcaaa

SEQ ID NO: 160 - DNA, 30 bp, synthetic construct
  source 1..30: mol_type = other DNA
aactggtggatgtcgtcaagctctcggaag